European Patent Application EP 4 737 565 A1, published May 6, 2026. Title: Utilization of sucrose for increased production of terpenes in Rhodobacter microbial cell factories. Applicant: Isobionics B.V. The sequence listing filed with the application follows.

SEQUENCE LISTING (11 sequences)

SEQ ID NO: 1 - DNA, 1434 bp, synthetic construct
  source 1..1434: mol_type = other DNA; note = nucleotide Inv_CO
atgacccagtcgcgcctccacgccgcccagaacgccctcgccaagctccacgagcaccgcggcaacaccttctacccgcacttccacctcgccccgccggccggctggatgaacgacccgaacggcctcatctggttcaacgaccgctaccacgccttctaccagcaccacccgatgtcggagcactggggcccgatgcactggggccacgccacctcggacgacatgatccactggcagcacgagccgatcgccctcgccccgggcgacgacaacgacaaggacggctgcttctcgggctcggccgtggacgacaacggcgtgctctcgctcatctacaccggccacgtgtggctcgacggcgccggcaacgacgacgccatccgcgaggtgcagtgcctcgccacctcgcgcgacggcatccacttcgagaagcagggcgtgatcctcaccccgccggagggcatcatgcacttccgcgacccgaaggtgtggcgcgaggccgacacctggtggatggtggtgggcgccaaggacccgggcaacaccggccagatcctcctctaccgcggctcgtcgctccgcgagtggaccttcgaccgcgtgctcgcccacgccgacgccggcgagtcgtacatgtgggagtgcccggacttcttctcgctcggcgaccagcactacctcatgttctcgccgcagggcatgaacgccgagggctactcgtaccgcaaccgcttccagtcgggcgtgatcccgggcatgtggtcgccgggccgcctcttcgcccagtcgggccacttcaccgagctcgacaacggccacgacttctacgccccgcagtcgttcctcgccaaggacggccgccgcatcgtgatcggctggatggacatgtgggagtcgccgatgccgtcgaagcgcgagggctgggccggctgcatgaccctcgcccgcgagctctcggagtcgaacggcaagctcctccagcgcccggtgcacgaggccgagtcgctccgccagcagcaccagtcggtgtcgccgcgcaccatctcgaacaagtacgtgctccaggagaacgcccaggccgtggagatccagctccagtgggccctcaagaactcggacgccgagcactacggcctccagctcggcaccggcatgcgcctctacatcgacaaccagtcggagcgcctcgtgctctggcgctactacccgcacgagaacctcgacggctaccgctcgatcccgctcccgcagcgcgacaccctcgccctccgcatcttcatcgacacctcgtcggtggaggtgttcatcaacgacggcgaggccgtgatgtcgtcgcgcatctacccgcagccggaggagcgcgagctctcgctctacgcctcgcacggcgtggccgtgctccagcacggcgccctctggctcctcggctga

SEQ ID NO: 2 - protein, 477 aa, synthetic construct
  source 1..477: note = protein Inv_CO
MTQSRLHAAQNALAKLHEHRGNTFYPHFHLAPPAGWMNDPNGLIWFNDRYHAFYQHHPMSEHWGPMHWGHATSDDMIHWQHEPIALAPGDDNDKDGCFSGSAVDDNGVLSLIYTGHVWLDGAGNDDAIREVQCLATSRDGIHFEKQGVILTPPEGIMHFRDPKVWREADTWWMVVGAKDPGNTGQILLYRGSSLREWTFDRVLAHADAGESYMWECPDFFSLGDQHYLMFSPQGMNAEGYSYRNRFQSGVIPGMWSPGRLFAQSGHFTELDNGHDFYAPQSFLAKDGRRIVIGWMDMWESPMPSKREGWAGCMTLARELSESNGKLLQRPVHEAESLRQQHQSVSPRTISNKYVLQENAQAVEIQLQWALKNSDAEHYGLQLGTGMRLYIDNQSERLVLWRYYPHENLDGYRSIPLPQRDTLALRIFIDTSSVEVFINDGEAVMSSRIYPQPEERELSLYASHGVAVLQHGALWLLG

SEQ ID NO: 3 - DNA, 915 bp, synthetic construct
  source 1..915: mol_type = other DNA; note = nucleotide Frk_CO
atgtcggccaaggtgtgggtgctcggcgacgccgtggtggacctcctcccggagtcggacggccgcctcctcccgtgcccgggcggcgccccggccaacgtggccgtgggcatcgcccgcctcggcggcacctcgggcttcatcggccgcgtgggcgacgacccgttcggcgccctcatgcagcgcaccctcctcaccgagggcgtggacatcacctacctcaagcaggacgagtggcaccgcacctcgaccgtgctcgtggacctcaacgaccagggcgagcgctcgttcaccttcatggtgcgcccgtcggccgacctcttcctcgagacgaccgacctcccgtgctggcgccacggcgagtggctccacctctgctcgatcgccctctcggccgagccgtcgcgcacctcggccttcaccgccatgaccgccatccgccacgccggcggcttcgtgtcgttcgacccgaacatccgcgaggacctctggcaggacgagcacctcctccgcctctgcctccgccaggccctccagctcgccgacgtggtgaagctctcggaggaggagtggcgcctcatctcgggcaagacccagaacgaccaggacatctgcgccctcgccaaggagtacgagatcgccatgctcctcgtgaccaagggcgccgagggcgtggtggtgtgctaccgcggccaggtgcaccacttcgccggcatgtcggtgaactgcgtggactcgaccggcgccggcgacgccttcgtggccggcctcctcaccggcctctcgtcgaccggcctctcgaccgacgagcgcgagatgcgccgcatcatcgacctcgcccagcgctgcggcgccctcgccgtgaccgccaagggcgccatgaccgccctcccgtgccgccaggagctcgagtga

SEQ ID NO: 4 - protein, 304 aa, synthetic construct
  source 1..304: note = protein Frk_CO
MSAKVWVLGDAVVDLLPESDGRLLPCPGGAPANVAVGIARLGGTSGFIGRVGDDPFGALMQRTLLTEGVDITYLKQDEWHRTSTVLVDLNDQGERSFTFMVRPSADLFLETTDLPCWRHGEWLHLCSIALSAEPSRTSAFTAMTAIRHAGGFVSFDPNIREDLWQDEHLLRLCLRQALQLADVVKLSEEEWRLISGKTQNDQDICALAKEYEIAMLLVTKGAEGVVVCYRGQVHHFAGMSVNCVDSTGAGDAFVAGLLTGLSSTGLSTDEREMRRIIDLAQRCGALAVTAKGAMTALPCRQELE

SEQ ID NO: 5 - DNA, 1248 bp, synthetic construct
  source 1..1248: mol_type = other DNA; note = nucleotide Trans_CO
atggccctcaacatcccgttccgcaacgcctactaccgcttcgcctcgtcgtactcgttcctcttcttcatctcgtggtcgctctggtggtcgctctacgccatctggctcaagggccacctcggcctcaccggcaccgagctcggcaccctctactcggtgaaccagttcacctcgatcctcttcatgatgttctacggcatcgtgcaggacaagctcggcctcaagaagccgctcatctggtgcatgtcgttcatcctcgtgctcaccggcccgttcatgatctacgtgtacgagccgctcctccagtcgaacttctcggtgggcctcatcctcggcgccctcttcttcggcctcggctacctcgccggctgcggcctcctcgactcgttcaccgagaagatggcccgcaacttccacttcgagtacggcaccgcccgcgcctggggctcgttcggctacgccatcggcgccttcttcgccggcatcttcttctcgatctcgccgcacatcaacttctggctcgtgtcgctcttcggcgccgtgttcatgatgatcaacatgcgcttcaaggacaaggaccaccagtgcgtggccgccgacgccggcggcgtgaagaaggaggacttcatcgccgtgttcaaggaccgcaacttctgggtgttcgtgatcttcatcgtgggcacctggtcgttctacaacatcttcgaccagcagctcttcccggtgttctactcgggcctcttcgagtcgcacgacgtgggcacccgcctctacggctacctcaactcgttccaggtggtgctcgaggccctctgcatggccatcatcccgttcttcgtgaaccgcgtgggcccgaagaacgccctcctcatcggcgtggtgatcatggccctccgcatcctctcgtgcgccctcttcgtgaacccgtggatcatctcgctcgtgaagctcctccacgccatcgaggtgccgctctgcgtgatctcggtgttcaagtactcggtggccaacttcgacaagcgcctctcgtcgaccatcttcctcatcggcttccagatcgcctcgtcgctcggcatcgtgctcctctcgaccccgaccggcatcctcttcgaccacgccggctaccagaccgtgttcttcgccatctcgggcatcgtgtgcctcatgctcctcttcggcatcttcttcctctcgaagaagcgcgagcagatcgtgatggagacgccggtgccgtcggccatctga

SEQ ID NO: 6 - protein, 415 aa, synthetic construct
  source 1..415: note = protein Trans_CO
MALNIPFRNAYYRFASSYSFLFFISWSLWWSLYAIWLKGHLGLTGTELGTLYSVNQFTSILFMMFYGIVQDKLGLKKPLIWCMSFILVLTGPFMIYVYEPLLQSNFSVGLILGALFFGLGYLAGCGLLDSFTEKMARNFHFEYGTARAWGSFGYAIGAFFAGIFFSISPHINFWLVSLFGAVFMMINMRFKDKDHQCVAADAGGVKKEDFIAVFKDRNFWVFVIFIVGTWSFYNIFDQQLFPVFYSGLFESHDVGTRLYGYLNSFQVVLEALCMAIIPFFVNRVGPKNALLIGVVIMALRILSCALFVNPWIISLVKLLHAIEVPLCVISVFKYSVANFDKRLSSTIFLIGFQIASSLGIVLLSTPTGILFDHAGYQTVFFAISGIVCLMLLFGIFFLSKKREQIVMETPVPSAI

SEQ ID NO: 7 - DNA, 87 bp, synthetic construct
  source 1..87: mol_type = other DNA; note = Pppa promoter
aaatttatttgctttgtgagcggataacaattattagattcaccggcgagccagcaggaatttcactctagatgacaggagggacat

SEQ ID NO: 8 - DNA, 12 bp, synthetic construct
  source 1..12: mol_type = other DNA; note = RBS
ggaggtgctgcc

SEQ ID NO: 9 - DNA, 250 bp, synthetic construct
  source 1..250: mol_type = other DNA; note = Prplm promoter
ggatgggcgtcaagggtcaagatgtcagaaggttcatcttgctcacgtcactgtgaggactttcacgtcgtcgtgacttgaggaaaggaaggacttatgattgagcgttcaagaaaataatgcgcttgcaggccacttgggcttacgataaggacaccgcttccgcgcacgcgtccgggccacaagtggcatgcccggccgtgcagagtctctgcaggatgcaggaccaatcgtttacggcgagggagat

SEQ ID NO: 10 - DNA, 1809 bp, synthetic construct
  source 1..1809: mol_type = other DNA; note = nucleotide zingiberene synthase
atggcccagaaggccaacacccagttcgacgccatctacttcaacggcgaggagaagaccgaggagaagggcgtgatccgccgcatgggcgagtaccacgccaacgtgtgggaccgcgacttcctcctctcgctctcgtcgccgtacggcgccccgtcgtacatggagcgcctcgagaccctcgtgaacgagatcaagatggacgtgttcatcaactcgctcctcgtgggcgacgaggagatcaacccgtcgtcgtacgacctcatcgagcgcttctcgatcgtggacgtggtgcagcgcctcggcatcgaccgccacttcgagaaggagatcaaggccgtgctcgactacacctaccgctactggtcggagaacggcatctcgtggcgccgcgagaacggcatcatcgacctctacaccaccgccctcggcttccgcatcctccgcctcaacggctactcggtgtcgccggacgtgttccacaacttcaaggacggcgacggccagttcgtgttcccgaccaagcagtcggacaaccagatccgcatcatgctctcgctctaccaggcctcggagatctcgttcccgggcgagtacatcatgcgcgaggccaaggagttctcgtacaagtacctcgaggaggccctcggcaagtggaagggcctcaacgagaagacccagctcatcgaggaggtggagtacatcatgaagtacccgtggcgctgccgcgtgccgcgctgggagacctggaactcgatcaagatcctccgccaggacatgggcgcctggatgctcatggagggcatctacaaggtgcagaacgagtggtcggagaagatcctcgaggtggccatcctcgacttcaacatcctccagtcgcaccaccacaacgagctcaagcacctcgccgagtggtgggacgaggccatcgtgaagcagctctcgttcttccgccaccgccacgtggagtattacttctggtacgcctgcggcctctacgagccggagtacgccgccacccgcctctgctacgccaagctcggcaccctcatcaccgtgatcgacgacatcttcgacacctacggcaccatcgacgagctcatcccgttccgcgaggccctcatccactgggacatgtcgatggtggaccagctcccgaactacatgcagatctcgctccagttcgcccgcaagacctacatggagatcgccatcgaggccgagaagatccacggcccgcacgtgcagaagtggatggaggactactggaagaccctcatctgggccgagttccaggacgccgagtggatcgccaagaactaccacccgaccctcatccagtacctcaagaactcgctcatctcgtcgaccgtgccggtggtgaccctcttcccgatgatcctcatcaacaccaacctcccgaacgacatcctcaacaaggtgaacaagttcgagtcgaaggtggcctggggctgccgcctcatcgacgactcgaaggacttccagcacgagcaggagcacggcgagaccgcctcgtggatcgagtgctacgtgcgcgacaacccgggcaccacccgcgagcaggccctcgaccacgtgaacatgctcatcgagctcaacatcgaggagctcaacaaggagcgcctcttcaacgagcacgacatcccgacctgctgcaagcgcctctacttcgactcgatgtaccgctcggtggccttcatctggcgcgacatcgacggcttcaccatctcgcaccagggcaccaaggacgacatcatgaagatcctcatcgagccgatctcgctctga

SEQ ID NO: 11 - protein, 602 aa, synthetic construct
  source 1..602: note = protein zingiberene synthase
MAQKANTQFDAIYFNGEEKTEEKGVIRRMGEYHANVWDRDFLLSLSSPYGAPSYMERLETLVNEIKMDVFINSLLVGDEEINPSSYDLIERFSIVDVVQRLGIDRHFEKEIKAVLDYTYRYWSENGISWRRENGIIDLYTTALGFRILRLNGYSVSPDVFHNFKDGDGQFVFPTKQSDNQIRIMLSLYQASEISFPGEYIMREAKEFSYKYLEEALGKWKGLNEKTQLIEEVEYIMKYPWRCRVPRWETWNSIKILRQDMGAWMLMEGIYKVQNEWSEKILEVAILDFNILQSHHHNELKHLAEWWDEAIVKQLSFFRHRHVEYYFWYACGLYEPEYAATRLCYAKLGTLITVIDDIFDTYGTIDELIPFREALIHWDMSMVDQLPNYMQISLQFARKTYMEIAIEAEKIHGPHVQKWMEDYWKTLIWAEFQDAEWIAKNYHPTLIQYLKNSLISSTVPVVTLFPMILINTNLPNDILNKVNKFESKVAWGCRLIDDSKDFQHEQEHGETASWIECYVRDNPGTTREQALDHVNMLIELNIEELNKERLFNEHDIPTCCKRLYFDSMYRSVAFIWRDIDGFTISHQGTKDDIMKILIEPISL